European Patent Application EP 4 137 516 A1, published February 22, 2023. Title: ANTIGEN-BINDING POLYPEPTIDES AGAINST CD39. Applicant: Universitätsklinikum Hamburg-Eppendorf. The sequence listing filed with the application follows.

SEQUENCE LISTING (113 sequences)

SEQ ID NO: 1 - protein, 9 aa, Vicugna pacos
  SITE 2: Xaa = Gly or Glu
  SITE 5: Xaa = Phe, Ser or Val
  SITE 6: Xaa = Ser or Asn
  SITE 7: Xaa = Phe or Ile
SXSIXXXNA

SEQ ID NO: 2 - protein, 6 aa, Vicugna pacos
  consensus CDR2
  SITE 6: Xaa = Asn, Ser, Tyr or Arg
ITSGGX

SEQ ID NO: 3 - protein, 14 aa, Vicugna pacos
  consensus CDR3
  SITE 10: Xaa = Asp or Glu
  SITE 12: Xaa = Pro or Tyr
  SITE 14: Xaa = Tyr, Asn or Ser
IGGSTWFGEXEXDX

SEQ ID NO: 4 - protein, 9 aa, Vicugna pacos
  CDR1 of clone SB24
SGSIFSFNA

SEQ ID NO: 5 - protein, 6 aa, Vicugna pacos
  CDR2 of clone SB24
ITSGGN

SEQ ID NO: 6 - protein, 14 aa, Vicugna pacos
  CDR3 of clone SB24
IGGSTWFGEDEPDY

SEQ ID NO: 7 - protein, 9 aa, Vicugna pacos
  CDR1 of clone SB27
SGSIFSFNA

SEQ ID NO: 8 - protein, 6 aa, Vicugna pacos
  CDR2 of clone SB27
ITSGGS

SEQ ID NO: 9 - protein, 14 aa, Vicugna pacos
  CDR3 of clone SB27
IGGSTWFGEDEYDY

SEQ ID NO: 10 - protein, 9 aa, Vicugna pacos
  CDR1 of clone SB28
SGSIFNFNA

SEQ ID NO: 11 - protein, 6 aa, Vicugna pacos
  CDR2 of clone SB28
ITSGGS

SEQ ID NO: 12 - protein, 14 aa, Vicugna pacos
  CDR3 of clone SB28
IGGSTWFGEEEYDY

SEQ ID NO: 13 - protein, 9 aa, Vicugna pacos
  CDR1 of clone SB130
SGSISSINA

SEQ ID NO: 14 - protein, 6 aa, Vicugna pacos
  CDR2 of clone SB130
ITSGGY

SEQ ID NO: 15 - protein, 14 aa, Vicugna pacos
  CDR3 of clone SB130
IGGSTWFGEDEYDN

SEQ ID NO: 16 - protein, 9 aa, Vicugna pacos
  CDR1 of clone SB131
SESIVSFNA

SEQ ID NO: 17 - protein, 6 aa, Vicugna pacos
  CDR2 of clone SB131
ITSGGR

SEQ ID NO: 18 - protein, 14 aa, Vicugna pacos
  CDR3 of clone SB131
IGGSTWFGEDEPDY

SEQ ID NO: 19 - protein, 9 aa, Vicugna pacos
  CDR1 of clone SB132
SGSIFNFNA

SEQ ID NO: 20 - protein, 6 aa, Vicugna pacos
  CDR2 of clone SB132
ITSGGS

SEQ ID NO: 21 - protein, 14 aa, Vicugna pacos
  CDR3 of clone SB132
IGGSTWFGEEEYDS

SEQ ID NO: 22 - protein, 9 aa, Vicugna pacos
  Consensus sequence - CDR1 - Family 2
  SITE 4: Xaa = Ile or Thr
  SITE 6: Xaa = Val or Ile
SGRXPXTTT

SEQ ID NO: 23 - protein, 7 aa, Vicugna pacos
  Consensus sequence - CDR2 - Family 2
  SITE 2: Xaa = Arg or Thr
  SITE 4: Xaa = Asn or Asp
  SITE 7: Xaa = Asn or Asp
IXWXSGX

SEQ ID NO: 24 - protein, 14 aa, Vicugna pacos
  Consensus sequence - CDR3 - Family 2
  SITE 6: Xaa = Leu, Ala or Asn
  SITE 7: Xaa = Pro or Leu
KYSRYXXQSTDYDY

SEQ ID NO: 25 - protein, 9 aa, Vicugna pacos
  CDR1 of clone SB128
SGRTPITTT

SEQ ID NO: 26 - protein, 7 aa, Vicugna pacos
  CDR2 of clone SB128
IRWDSGN

SEQ ID NO: 27 - protein, 14 aa, Vicugna pacos
  CDR3 of clone SB128
KYSRYLPQSTDYDY

SEQ ID NO: 28 - protein, 9 aa, Vicugna pacos
  CDR1 of clone SB126
SGRIPVTTT

SEQ ID NO: 29 - protein, 7 aa, Vicugna pacos
  CDR2 of clone SB126
IRWNSGD

SEQ ID NO: 30 - protein, 14 aa, Vicugna pacos
  CDR3 of clone SB126
KYSRYAPQSTDYDY

SEQ ID NO: 31 - protein, 9 aa, Vicugna pacos
  CDR1 of clone SB127
SGRIPVTTT

SEQ ID NO: 32 - protein, 7 aa, Vicugna pacos
  CDR2 of clone SB127
ITWNSGN

SEQ ID NO: 33 - protein, 14 aa, Vicugna pacos
  CDR3 of clone SB127
KYSRYNLQSTDYDY

SEQ ID NO: 34 - protein, 9 aa, Vicugna pacos
  CDR1 of clone SB129
SGRTPITTT

SEQ ID NO: 35 - protein, 7 aa, Vicugna pacos
  CDR2 of clone SB129
IRWNSGD

SEQ ID NO: 36 - protein, 14 aa, Vicugna pacos
  CDR3 of clone SB129
KYSRYAPQSTDYDY

SEQ ID NO: 37 - protein, 517 aa, Homo sapiens
  human CD39 protein sequence
MKGTKDLTSQQKESNVKTFCSKNILAILGFSSIIAVIALLAVGLTQNKALPENVKYGIVLDAGSSHTSLYIYKWPAEKENDTGVVHQVEECRVKGPGISKFVQKVNEIGIYLTDCMERAREVIPRSQHQETPVYLGATAGMRLLRMESEELADRVLDVVERSLSNYPFDFQGARIITGQEEGAYGWITINYLLGKFSQKTRWFSIVPYETNNQETFGALDLGGASTQVTFVPQNQTIESPDNALQFRLYGKDYNVYTHSFLCYGKDQALWQKLAKDIQVASNEILRDPCFHPGYKKVVNVSDLYKTPCTKRFEMTLPFQQFEIQGIGNYQQCHQSILELFNTSYCPYSQCAFNGIFLPPLQGDFGAFSAFYFVMKFLNLTSEKVSQEKVTEMMKKFCAQPWEEIKTSYAGVKEKYLSEYCFSGTYILSLLLQGYHFTADSWEHIHFIGKIQGSDAGWTLGYMLNLTNMIPAEQPLSTPLSHSTYVFLMVLFSLVLFTVAIIGLLIFHKPSYFWKDMV

SEQ ID NO: 38 - protein, 122 aa, Vicugna pacos
  Clone SB24
QVQLVESGGGLVQPGGSLRLSCAASGSIFSFNAMGWYRQAPGKQRELVAAITSGGNTNYADSVKGRFAISRDNAKNTVYLQMSSLKPEDTAVYYCKGIGGSTWFGEDEPDYWGQGTQVTVSS

SEQ ID NO: 39 - protein, 122 aa, Vicugna pacos
  Clone SB27
QVQLVESGGGLVQPGGSLRLSCAASGSIFSFNAMGWYRQAPGKQRELVAAITSGGSTNYADSVKGRFTISRDNAKNTVYLQMNSLKPEDTAVYYCNGIGGSTWFGEDEYDYWGQGTQVTVSS

SEQ ID NO: 40 - protein, 122 aa, Vicugna pacos
  Clone SB28
QVQLVESGGGLVQPGGSLRLSCAASGSIFNFNAMGWYRQAPGKQRELVAAITSGGSTNYADSVKGRFTISRDNAKNTVYLQMNSLKPEDTAVYYCHGIGGSTWFGEEEYDYWGQGTQVTVSS

SEQ ID NO: 41 - protein, 122 aa, Vicugna pacos
  Clone SB130
QVQLVESGGGSVQPGGSLKLSCAASGSISSINAMGWYRQAPGKQRELVAAITSGGYTNYADSVKGRFTISRDNAKNTVYLQMNSLKPEDTAVYYCNAIGGSTWFGEDEYDNWGQGTQVTVSS

SEQ ID NO: 42 - protein, 122 aa, Vicugna pacos
  Clone SB131
QVQLVESGGGLVQPGGSLRLSCAASESIVSFNAMGWYRQAPGKQRDLVAAITSGGRTNYAESVKGRFTISRDDAKNTVYLQMNSLKPEDTAVYYCHAIGGSTWFGEDEPDYWGQGTQVTVSS

SEQ ID NO: 43 - protein, 122 aa, Vicugna pacos
  Clone SB132
QVQLVESGGGLVQPGGSLRLSCAASGSIFNFNAMGWYRQASGKQRELVAAITSGGSTNYADSVKGRFTISRGNAKNTVYLQMNSLKPEDTAVYYCHGIGGSTWFGEEEYDSWGQGTQVTVSS

SEQ ID NO: 44 - protein, 123 aa, Vicugna pacos
  Clone SB128
QVQLVESGGGLVQAGDSLRLSCAASGRTPITTTTGWFRQAPGKEREFVAAIRWDSGNTNYADSAKGRFTISRDSAKNLLYLQMTNLKPEDTAVYYCAAKYSRYLPQSTDYDYWGQGTQVTVSS

SEQ ID NO: 45 - protein, 123 aa, Vicugna pacos
  Clone SB126
QVQLVESGGGLVQAGDSLRLSCAASGRIPVTTTTAWFRQAPGKEREFVAAIRWNSGDAAYADSAKGRFTISRDSAKNTLYLQMNNLEPEDTAVYYCAAKYSRYAPQSTDYDYWGQGTQVTVSS

SEQ ID NO: 46 - protein, 123 aa, Vicugna pacos
  Clone SB127
QVQLVESGGGLVQAGDSLRLSCAASGRIPVTTTTAWFRQAPGKEREFVAAITWNSGNTNYADSAKGRFTISRDSAKNTLYLQMNNLKPEDTAVYYCAAKYSRYNLQSTDYDYWGQGTQVTVSS

SEQ ID NO: 47 - protein, 123 aa, Vicugna pacos
  Clone SB129
QVQLVESGGGLVQAGDSLRLSCAASGRTPITTTTGWFRQAPGKEREFVAAIRWNSGDAAYADSAKGRFTISRDSAKNTLYLQMNNLEPEDTAVYYCAAKYSRYAPQSTDYDYWGQGTQVTVSS

SEQ ID NO: 48 - protein, 9 aa, Vicugna pacos
  SITE 1: Xaa = Ser or Thr
  Consensus sequence - CDR1 - Family 10
  SITE 5: Xaa = Ser, Lys, Thr or Asn
  SITE 6: Xaa = Thr or Ile
  SITE 7: Xaa = His, Asn, Tyr or Gln
XKRTXXXYA

SEQ ID NO: 49 - protein, 7 aa, Vicugna pacos
  Consensus sequence - CDR2 - Family 10
INWNGGT

SEQ ID NO: 50 - protein, 14 aa, Vicugna pacos
  Consensus sequence - CDR3 - Family 10
  SITE 2: Xaa = Val, Ile or Leu
  SITE 7: Xaa = Leu, Tyr or Thr
  SITE 8: Xaa = Thr or Ser
  SITE 10: Xaa = Asn, Arg, Lys or Thr
  SITE 11: Xaa = Glu or Asp
  SITE 13: Xaa = Gln or His
  SITE 14: Xaa = His, Tyr or Val
KXDGLGXXSXXYXX

SEQ ID NO: 51 - protein, 9 aa, Vicugna pacos
  CDR1 of clone SB32
SKRTSTHYA

SEQ ID NO: 52 - protein, 7 aa, Vicugna pacos
  CDR2 of clone SB32
INWNGGT

SEQ ID NO: 53 - protein, 14 aa, Vicugna pacos
  CDR3 of clone SB32
KVDGLGLTSNEYQH

SEQ ID NO: 54 - protein, 9 aa, Vicugna pacos
  CDR1 of clone SB34
SKRTKTNYA

SEQ ID NO: 55 - protein, 7 aa, Vicugna pacos
  CDR2 of clone SB34
INWNGGT

SEQ ID NO: 56 - protein, 14 aa, Vicugna pacos
  CDR3 of clone SB34
KVDGLGYTSREYQY

SEQ ID NO: 57 - protein, 9 aa, Artificial Sequence
  CDR1 of clone SB33
SKRTTTQYA

SEQ ID NO: 58 - protein, 7 aa, Artificial Sequence
  CDR2 of clone SB33
INWNGGT

SEQ ID NO: 59 - protein, 14 aa, Artificial Sequence
  CDR3 of clone SB33
KVDGLGTSSNEYQH

SEQ ID NO: 60 - protein, 9 aa, Artificial Sequence
  CDR1 of clone SB30
SKRTSTQYA

SEQ ID NO: 61 - protein, 7 aa, Artificial Sequence
  CDR2 of clone SB30
INWNGGT

SEQ ID NO: 62 - protein, 14 aa, Artificial Sequence
  CDR3 of clone SB30
KVDGLGLTSNEYQH

SEQ ID NO: 63 - protein, 9 aa, Artificial Sequence
  CDR1 of clone SB31
SKRTSINYA

SEQ ID NO: 64 - protein, 7 aa, Artificial Sequence
  CDR2 of clone SB31
INWNGGT

SEQ ID NO: 65 - protein, 14 aa, Artificial Sequence
  CDR3 of clone SB31
KVDGLGYTSNEYHY

SEQ ID NO: 66 - protein, 9 aa, Artificial Sequence
  CDR1 of clone SB168
SKRTNTYYA

SEQ ID NO: 67 - protein, 7 aa, Artificial Sequence
  CDR2 of clone SB168
INWNGGT

SEQ ID NO: 68 - protein, 14 aa, Artificial Sequence
  CDR3 of clone SB168
KVDGLGTTSNEYQY

SEQ ID NO: 69 - protein, 9 aa, Artificial Sequence
  CDR1 of clone SB169
SKRTSTNYA

SEQ ID NO: 70 - protein, 7 aa, Artificial Sequence
  CDR2 of clone SB169
INWNGGT

SEQ ID NO: 71 - protein, 14 aa, Artificial Sequence
  CDR3 of clone SB169
KVDGLGYTSNEYQH

SEQ ID NO: 72 - protein, 9 aa, Artificial Sequence
  CDR1 of clone SB175
SKRTSTNYA

SEQ ID NO: 73 - protein, 7 aa, Artificial Sequence
  CDR2 of clone SB175
INWNGGT

SEQ ID NO: 74 - protein, 14 aa, Artificial Sequence
  CDR3 of clone SB175
KVDGLGYTSKEYQV

SEQ ID NO: 75 - protein, 9 aa, Artificial Sequence
  CDR1 of clone SB170
SKRTTTHYA

SEQ ID NO: 76 - protein, 7 aa, Artificial Sequence
  CDR2 of clone SB170
INWNGGT

SEQ ID NO: 77 - protein, 14 aa, Artificial Sequence
  CDR3 of clone SB170
KVDGLGYTSNEYQY

SEQ ID NO: 78 - protein, 9 aa, Artificial Sequence
  CDR1 of clone SB171
SKRTSTQYA

SEQ ID NO: 79 - protein, 7 aa, Artificial Sequence
  CDR2 of clone SB171
INWNGGT

SEQ ID NO: 80 - protein, 14 aa, Artificial Sequence
  CDR3 of clone SB171
KVDGLGTTSNEYQH

SEQ ID NO: 81 - protein, 9 aa, Artificial Sequence
  CDR1 of clone SB172
SKRTSTQYA

SEQ ID NO: 82 - protein, 7 aa, Artificial Sequence
  CDR2 of clone SB172
INWNGGT

SEQ ID NO: 83 - protein, 14 aa, Artificial Sequence
  CDR3 of clone SB172
KIDGLGTTSNDYQH

SEQ ID NO: 84 - protein, 9 aa, Artificial Sequence
  CDR1 of clone SB173
TKRTSTNYA

SEQ ID NO: 85 - protein, 7 aa, Artificial Sequence
  CDR2 of clone SB173
INWNGGT

SEQ ID NO: 86 - protein, 14 aa, Artificial Sequence
  CDR3 of clone SB173
KIDGLGYTSTEYQY

SEQ ID NO: 87 - protein, 9 aa, Artificial Sequence
  CDR1 of clone SB174
TKRTTTHYA

SEQ ID NO: 88 - protein, 7 aa, Artificial Sequence
  CDR2 of clone SB174
INWNGGT

SEQ ID NO: 89 - protein, 14 aa, Artificial Sequence
  CDR3 of clone SB174
KVDGLGYTSTEYQY

SEQ ID NO: 90 - protein, 9 aa, Artificial Sequence
  CDR1 of clone SB176
SKRTSTNYA

SEQ ID NO: 91 - protein, 7 aa, Artificial Sequence
  CDR2 of clone SB176
INWNGGT

SEQ ID NO: 92 - protein, 14 aa, Artificial Sequence
  CDR3 of clone SB176
KLDGLGYTSNEYHY

SEQ ID NO: 93 - protein, 123 aa, Vicugna pacos
  Clone SB32
QVQLVESGGGLVQAGGSLRLSCAVSKRTSTHYAMGWFRQAPGLVREFVGVINWNGGTTYYADSVKGRFFISRDNAKNTMALQMNNLKPEDTAVYYCALKVDGLGLTSNEYQHWGQGTQVTVSS

SEQ ID NO: 94 - protein, 123 aa, Vicugna pacos
  Clone SB34
QVQLVESGGGLVQAGGSLRLSCAVSKRTKTNYAMGWFRQAPGEVREFVGVINWNGGTTYYADSVKGRFTMSRDNAKNTIYLQMNNLKPEDTAVYYCALKVDGLGYTSREYQYWGQGTQVTVSS

SEQ ID NO: 95 - protein, 123 aa, Vicugna pacos
  Clone SB33
QVQLVESGGGLVQAGASLRLSCAVSKRTTTQYAMGWFRQAPGLVREFVAVINWNGGTTYYADSVKGRFTISRDNAKNTMYLQMNNLKPEDTAVYYCALKVDGLGTSSNEYQHWGQGTQVTVSS

SEQ ID NO: 96 - protein, 112 aa, Vicugna pacos
  Clone SB30
QVQLVESGGGLVQAGGSLRLSCAVSKRTSTQYAMGWFRQAPGLVREFVAVINWNGGTTYYADSVKGRFTISRDNAKNTMYLQMNNLKPEDTAVYYCALKVDGLGLTSNEYQH

SEQ ID NO: 97 - protein, 123 aa, Vicugna pacos
  Clone SB31
QVQLVESGGGLVQAGGSLRLSCVVSKRTSINYAMGWFRQAPGEVREFVGLINWNGGTTYYADSVKGRFTISRDNAKNTIYLQMNNLKPEDTAVYYCALKVDGLGYTSNEYHYWGQGTQVTVSS

SEQ ID NO: 98 - protein, 123 aa, Vicugna pacos
  Clone SB168
QVQLVESGGGLVQAGGSLRLSCAVSKRTNTYYAMGWFRQAPGEVREFVAVINWNGGTTYYADSVKGRFTISRDNAKNMIYLQMNNLKPEDTAVYYCALKVDGLGTTSNEYQYWGQGTQVTVSS

SEQ ID NO: 99 - protein, 123 aa, Vicugna pacos
  Clone SB169
QVQLVESGGGLVQAGGSLRLSCAVSKRTSTNYAMGWFRQAPGLVREFVALINWNGGTTYYSDSVKGRFTISRDNAKNTMYLQMNNLKPEDTAVYYCALKVDGLGYTSNEYQHWGQGTQVTVSS

SEQ ID NO: 100 - protein, 112 aa, Vicugna pacos
  Clone SB175
QVQLVESGGGLVQAGGSLRLSCAVSKRTSTNYAMGWFRQAPGLVREFVALINWNGGTTYYSDSVKGRFTISRDNAKNTMALQMNNLKPEDTAVYYCALKVDGLGYTSKEYQV

SEQ ID NO: 101 - protein, 123 aa, Vicugna pacos
  Clone SB170
QVQLVESGGGLVQAGGSLRLSCAVSKRTTTHYAMGWFRQAPGEVREFVAVINWNGGTTYYADSVKGRFTVSRDNAKNTIYLQMNNLKPEDTALYYCALKVDGLGYTSNEYQYWGQGTQVTVSS

SEQ ID NO: 102 - protein, 123 aa, Vicugna pacos
  Clone SB171
QVQLVESGGGLVQAGGSLRLSCAVSKRTSTQYAMGWFRQAPGLVREFVAVINWNGGTTYYADSVKGRFTISRDNAKNTMYLQMNNLKPEDTAVYYCALKVDGLGTTSNEYQHWGQGTQVTVSS

SEQ ID NO: 103 - protein, 123 aa, Vicugna pacos
  Clone SB172
QVQLVESGGGLVQAGGSLRLSCAVSKRTSTQYAMGWFRQAPGLVREFVAVINWNGGTTYYADSVKGRFTISRDNAKNTMYLQMNNLKPEDTAVYYCALKIDGLGTTSNDYQHWGQGTQVTVSS

SEQ ID NO: 104 - protein, 123 aa, Vicugna pacos
  Clone SB173
QVQLVESGGGLVQAGGSLRLSCAVTKRTSTNYAMGWFRQAPGEVREFVGVINWNGGTTYYADSVKGRFTISRDNAKNTLYLQMGDLKPEDTALYYCALKIDGLGYTSTEYQYWGQGTQVTVSS

SEQ ID NO: 105 - protein, 123 aa, Vicugna pacos
  Clone SB174
QVQLVESGGGLVQAGGSLRLSCAVTKRTTTHYAMGWFRQAPGEVREFVGVINWNGGTTYYADSVKGRFTISRDNAKNTIYLQMNNLKPEDTAVYYCALKVDGLGYTSTEYQYWGPGDPGHRLL

SEQ ID NO: 106 - protein, 123 aa, Vicugna pacos
  Clone SB176
QVQLVESGGGLVQAGGSLRLSCVVSKRTSTNYAMGWFRQAPGEVREFVGLINWNGGTTYYADSVKGRFTISRDNAKSTMNLQMNNLKPEDTAVYYCALKLDGLGYTSNEYHYWGQGTQVTVSS

SEQ ID NO: 107 - protein, 113 aa, Vicugna pacos
  Clone SB134
QVKLQESGGGWVQPGGSLRLSCAASGFTFRTHFMSWVRQAPGQGLEWVSGITSGGRTSYVDSVKGRFTISRDNAANTLYLQMNSLKPEDTAVYFCTKGDSGARGQGTQVTVSS

SEQ ID NO: 108 - protein, 124 aa, Vicugna pacos
  Clone SB135
QVKLQESGGGLVQAGGSLRLSCTASEESFNKYGVGWFRQAPGKERAFVVAIRPSGVITSYADSVKGRFTISRDSAKNTAYLQMNSLKPEDTALYYCAANSRNTNYYRPNGYDYWGRGTQVTVSS

SEQ ID NO: 109 - protein, 120 aa, Vicugna pacos
  Clone SB136
DVQLQASGGGLVQPGGSLRLSCAASGFRFSIYDMSWVRRPPGKGLEWVSSITSPGGTTYADSVKGRFTISRDNDKNTLYLQMNSLKPEDTAIYYCAKAYGGRSVVAQTARGQGTQVTVSS

SEQ ID NO: 110 - protein, 126 aa, Vicugna pacos
  Clone SB137
QVKLQESGGGLGQAGGSLRLSCSASARTSATYVMGWFRQAPGKEREFVATISRSTSTTYYGDSVKGRFTISRDNAKNAVYLQMNSLKPEDTAVYYCATRAPRYGTASTRLSDYDNWGQGTQVTVSS

SEQ ID NO: 111 - protein, 119 aa, Vicugna pacos
  Clone SB39
QVQLVESGGGLVQPGGSLRLSCAASGFTLDYFAIGWFRQGPGKERDWVSCISKDGTTYYIDSVKGRFTISRDNAKNTGYLQMSGLKPDDTAVYYCARGAGGCQSDFGARGQGTQVTVSS

SEQ ID NO: 112 - protein, 124 aa, Vicugna pacos
  Clone SB90
QVQLVESGGGLVQAGGSLRLSCAVSGLNNYAIGWLRQAPGKEREGVSCINCFDDFTYYADSVKGRFTVSCDNANHTVNLEMNSLRPEDTAVYYCAAGTCGSWWRYTPTPADGAWGRGTQVTVSS

SEQ ID NO: 113 - protein, 123 aa, Vicugna pacos
  Clone SB112
QVQLQESGGGLVQAGGSLRLSCTASGRSFSSNAMGWFRQAPGKEREFVARINWSGSRTFYTDSVKGRFTISRDNAKNTMYLQMNSLKPEDTAVYYCAADPNYGSSITSGYTYWGQGTQVTVSS